European Patent Specification EP 3 416 659 B1, published June 5, 2024. Title: Prevention of graft rejection by prior use of modified grafts. Applicant: Fraunhofer-Gesellschaft zur Förderung der angewandten Forschung e.V. The sequence listing filed with the application follows.

SEQUENCE LISTING (21 sequences)

SEQ ID NO: 1 - DNA, 360 bp, Artificial Sequence
  Mouse Anti-CD4 Heavy Chain
  CDS (1)..(360)
gaggttcagctccagcagtctgggactgtgctggcaaggcctggggcttccgtgcagatgtcctgcaaggcttctggctacagctttgccaactactggatgcactgggtaaaacagaggcctggacagggtctacaatggattggtgctctttatcctggaaatgttgatactacctacaaccagaagttcaaggacaaggccaaactgactgcagtcacatccgccagcactgcctacatggagctcagcagcctgacaaatgaggactctgcggtctattactgtacaagaatgggtactactttagaagccccccttgactattggggccaaggcaccactctcacagtctcctca

SEQ ID NO: 2 - protein, 120 aa, Artificial Sequence
  Synthetic Construct
EVQLQQSGTVLARPGASVQMSCKASGYSFANYWMHWVKQRPGQGLQWIGALYPGNVDTTYNQKFKDKAKLTAVTSASTAYMELSSLTNEDSAVYYCTRMGTTLEAPLDYWGQGTTLTVSS

SEQ ID NO: 3 - DNA, 360 bp, Artificial Sequence
  Heavy chain VH4
  CDS (1)..(360)
gaggttcagctccagcagtctgggactgagctgaaaaggcctggggcttccgtgaagatgtcctgcaaggcttctggctacacctttgccaactactggatgcactgggtaaaacaggcccctggacagggtctacaatggattggtgctctttatcctggaaatgttgatactacctacaaccagaagttcaaggacaaggccaaactgactgcagtcacatccgccagcactgcctacatggagctcagcagcctgacaaatgaggactctgcggtctattactgtacaagaatgggtactactttagaagccccccttgactattggggccaaggcaccactgtcacagtctcctca

SEQ ID NO: 4 - protein, 120 aa, Artificial Sequence
  Synthetic Construct
EVQLQQSGTELKRPGASVKMSCKASGYTFANYWMHWVKQAPGQGLQWIGALYPGNVDTTYNQKFKDKAKLTAVTSASTAYMELSSLTNEDSAVYYCTRMGTTLEAPLDYWGQGTTVTVSS

SEQ ID NO: 5 - DNA, 360 bp, Artificial Sequence
  Heavy chain VH3
  CDS (1)..(360)
gaggttcagctccagcagtctgggtctgagctgaaaaggcctggggcttccgtgaagatgtcctgcaaggcttctggctacacctttgccaactactggatgcactgggtaaaacaggcccctggacagggtctacaatggattggtgctctttatcctggaaatgttgatactacctacaaccagaagttcaaggacaaggccaaactgactgcagtcacatccgccagcactgcctacatggagctcagcagcctgacaaatgaggacaccgcggtctattactgtacaagaatgggtactactttagaagccccccttgactattggggccaaggcacccttgtcacagtctcctca

SEQ ID NO: 6 - protein, 120 aa, Artificial Sequence
  Synthetic Construct
EVQLQQSGSELKRPGASVKMSCKASGYTFANYWMHWVKQAPGQGLQWIGALYPGNVDTTYNQKFKDKAKLTAVTSASTAYMELSSLTNEDTAVYYCTRMGTTLEAPLDYWGQGTLVTVSS

SEQ ID NO: 7 - DNA, 360 bp, Artificial Sequence
  Heavy chain VH2
  CDS (1)..(360)
gaggttcagctccagcagtctgggtctgagctgaaaaggcctggggcttccgtgaaggtgtcctgcaaggcttctggctacacctttgccaactactggatgcactgggtaaaacaggcccctggacagggtctacaatggattggtgctctttatcctggaaatgttgatactacctacaaccagaagttcaaggacaaggccaaactgactgcagacacatccgccagcactgcctacatggagctcagcagcctgacaaatgaggacaccgcggtctattactgtacaagaatgggtactactttagaagccccccttgactattggggccaaggcacccttgtcacagtctcctca

SEQ ID NO: 8 - protein, 120 aa, Artificial Sequence
  Synthetic Construct
EVQLQQSGSELKRPGASVKVSCKASGYTFANYWMHWVKQAPGQGLQWIGALYPGNVDTTYNQKFKDKAKLTADTSASTAYMELSSLTNEDTAVYYCTRMGTTLEAPLDYWGQGTLVTVSS

SEQ ID NO: 9 - DNA, 360 bp, Artificial Sequence
  Heavy chain VH1
  CDS (1)..(360)
gaggttcagctccagcagtctgggtctgagctgaaaaggcctggggcttccgtgaaggtgtcctgcaaggcttctggctacacctttgccaactactggatgcactgggtaagacaggcccctggacagggtctacaatggattggtgctctttatcctggaaatgttgatactacctacaaccagaagttcaaggacaaggccaaaatcactagagacacatccgccagcactgcctacatggagctcagcagcctgacaaatgaggacaccgcggtctattactgtacaagaatgggtactactttagaagccccccttgactattggggccaaggcacccttgtcacagtctcctca

SEQ ID NO: 10 - protein, 120 aa, Artificial Sequence
  Synthetic Construct
EVQLQQSGSELKRPGASVKVSCKASGYTFANYWMHWVRQAPGQGLQWIGALYPGNVDTTYNQKFKDKAKITRDTSASTAYMELSSLTNEDTAVYYCTRMGTTLEAPLDYWGQGTLVTVSS

SEQ ID NO: 11 - DNA, 318 bp, Artificial Sequence
  Mouse Anti-CD4 Light Chain
  CDS (1)..(318)
caaattgttctcacccagtctccagcaatcatgtctgcatctccaggggagaaggtcgccatgacctgcagtgccaggtcaagtgtaagttacttgtactggtaccagcagaagccaggatcctcccccagactcctgatttatgacacatccaacctggcttctggagtccctgttcgcttcattggcagtgggtctgggacctcttactctctcacaatcagccgaatggaggctgaagatgctgccacttattactgccagcagtggagtgattacccgctcacgttcggtgctgggaccaagctggagctgaaa

SEQ ID NO: 12 - protein, 106 aa, Artificial Sequence
  Synthetic Construct
QIVLTQSPAIMSASPGEKVAMTCSARSSVSYLYWYQQKPGSSPRLLIYDTSNLASGVPVRFIGSGSGTSYSLTISRMEAEDAATYYCQQWSDYPLTFGAGTKLELK

SEQ ID NO: 13 - DNA, 318 bp, Artificial Sequence
  Light Chain VK4
  CDS (1)..(318)
caaattgttctcacccagtctccagcaatcctgtctgcatctccaggggagaaggccgccatgacctgcagtgccaggtcaagtgtaagttacttgtactggtaccagcagaagccagggtcctcccccagactcctgatttatgacacatccaacctggcttctggagtcccttctcgcttcattggcagtgggtctgggaccgattactctctcacaatcagcagcatggaggctgaagatgctgccacttattactgccagcagtggagtgattacccgctcacgttcggtgctgggaccaagctggagatcaaa

SEQ ID NO: 14 - protein, 106 aa, Artificial Sequence
  Synthetic Construct
QIVLTQSPAILSASPGEKAAMTCSARSSVSYLYWYQQKPGSSPRLLIYDTSNLASGVPSRFIGSGSGTDYSLTISSMEAEDAATYYCQQWSDYPLTFGAGTKLEIK

SEQ ID NO: 15 - DNA, 318 bp, Artificial Sequence
  Light chain VK3
  CDS (1)..(318)
caaattgttctcacccagtctccagcaaccctgtctgcatctccaggggagaaggccgccatgacctgcagtgccaggtcaagtgtaagttacttgtactggtaccagcagaagccagggtcctcccccagactcctgatttatgacacatccaacctggcttctggagtcccttctcgcttcattggcagtgggtctgggaccgattactctctcacaatcagcagcatggaggctgaagatgctgccacttattactgccagcagtggagtgattacccgctcacgttcggtgctgggaccaagctggagatcaaa

SEQ ID NO: 16 - protein, 106 aa, Artificial Sequence
  Synthetic Construct
QIVLTQSPATLSASPGEKAAMTCSARSSVSYLYWYQQKPGSSPRLLIYDTSNLASGVPSRFIGSGSGTDYSLTISSMEAEDAATYYCQQWSDYPLTFGAGTKLEIK

SEQ ID NO: 17 - DNA, 318 bp, Artificial Sequence
  Light chain VK2
  CDS (1)..(318)
caaattgttctcacccagtctccagcaaccctgtctgcatctccaggggagaaggccgccatgacctgcagtgccaggtcaagtgtaagttacttgtactggtaccagcagaagccagggtcctcccccagactcctgatttatgacacatccaacctggcttctggagtcccttctcgcttcagcggcagtgggtctgggaccgattactctctcacaatcagcagcatggaggctgaagatgctgccacttattactgccagcagtggagtgattacccgctcacgttcggtgctgggaccaagctggagatcaaa

SEQ ID NO: 18 - protein, 106 aa, Artificial Sequence
  Synthetic Construct
QIVLTQSPATLSASPGEKAAMTCSARSSVSYLYWYQQKPGSSPRLLIYDTSNLASGVPSRFSGSGSGTDYSLTISSMEAEDAATYYCQQWSDYPLTFGAGTKLEIK

SEQ ID NO: 19 - DNA, 318 bp, Artificial Sequence
  Light chain VK1
  CDS (1)..(318)
caaattgttctcacccagtctccagcaaccctgtctgcatctccaggggagaaggccgccatgacctgcagtgccaggtcaagtgtaagttacttgtactggtaccagcagaagccagggtcctcccccagagccctgatttatgacacatccaacctggcttctggagtcccttctcgcttcagcggcagtgggtctgggaccgattactctctcacaatcagcagcatggaggctgaagatgctgccacttattactgccagcagtggagtgattacccgctcacgttcggtgctgggaccaagctggagatcaaa

SEQ ID NO: 20 - protein, 106 aa, Artificial Sequence
  Synthetic Construct
QIVLTQSPATLSASPGEKAAMTCSARSSVSYLYWYQQKPGSSPRALIYDTSNLASGVPSRFSGSGSGTDYSLTISSMEAEDAATYYCQQWSDYPLTFGAGTKLEIK

SEQ ID NO: 21 - protein, 7 aa, Artificial
  cyclic peptide
CNSNQIC